European Patent Specification EP 3 684 415 B1, published July 8, 2026. Title: METHODS OF REDUCING PARTICLE FORMATION AND COMPOSITIONS FORMED THEREBY. Applicant: Regeneron Pharmaceuticals, Inc. The sequence listing filed with the application follows.

SEQUENCE LISTING (31 sequences)

SEQ ID NO: 1 - protein, 17 aa, Cricetulus griseus
DLLVAHNTWNSYQNMLR

SEQ ID NO: 2 - protein, 22 aa, Cricetulus griseus
LIRYNNFLHDPLSLCEACIPKP

SEQ ID NO: 3 - protein, 12 aa, Cricetulus griseus
SVLLDAASGQLR

SEQ ID NO: 4 - protein, 13 aa, Cricetulus griseus
DQSLVEDMNSMVR

SEQ ID NO: 5 - protein, 17 aa, Cricetulus griseus
QFNSGTYNNQWMIVDYK

SEQ ID NO: 6 - protein, 20 aa, Cricetulus griseus
QGPQEAYPLIAGNNLVFSSY

SEQ ID NO: 7 - protein, 19 aa, Cricetulus griseus
SMLHMGQPDLWTFSPISVP

SEQ ID NO: 8 - protein, 21 aa, Cricetulus griseus
YNNFLHDPLSLCEACIPKPNA

SEQ ID NO: 9 - protein, 13 aa, Cricetulus griseus
LALDGATWADIFK

SEQ ID NO: 10 - protein, 13 aa, Cricetulus griseus
LSLGSGSCSAIIK

SEQ ID NO: 11 - protein, 13 aa, Cricetulus griseus
YVQPQGCVLEWIR

SEQ ID NO: 12 - protein, 19 aa, Cricetulus griseus
RMSMLAASGPTWDQLPPFQ

SEQ ID NO: 13 - protein, 12 aa, Cricetulus griseus
SFLEINLEWMQR

SEQ ID NO: 14 - protein, 22 aa, Cricetulus griseus
VLTILEQIPGMVVVADADKTED

SEQ ID NO: 15 - protein, 14 aa, Cricetulus griseus
VRSVLLDAASGQLR

SEQ ID NO: 16 - protein, 16 aa, Cricetulus griseus
LTLLQLKGLEDSYEGR

SEQ ID NO: 17 - protein, 18 aa, Cricetulus griseus
MSMLAASGPTWDQLPPFQ

SEQ ID NO: 18 - protein, 9 aa, Cricetulus griseus
VTSFSLAKR

SEQ ID NO: 19 - protein, 9 aa, Cricetulus griseus
QNLDPPVSR

SEQ ID NO: 20 - protein, 10 aa, Cricetulus griseus
IIKKYQLQFR

SEQ ID NO: 21 - protein, 19 aa, Cricetulus griseus
AQIFQRDQSLVEDMNSMVR

SEQ ID NO: 22 - protein, 22 aa, Cricetulus griseus
LIRYNNFLHDPLSLCEACIPKP

SEQ ID NO: 23 - protein, 12 aa, Cricetulus griseus
SVLLDAASGQLR

SEQ ID NO: 24 - protein, 13 aa, Cricetulus griseus
DQSLVEDMNSMVR

SEQ ID NO: 25 - protein, 17 aa, Cricetulus griseus
DLLVAHNTWNSYQNMLR

SEQ ID NO: 26 - protein, 21 aa, Cricetulus griseus
YNNFLHDPLSLCEACIPKPNA

SEQ ID NO: 27 - protein, 19 aa, Cricetulus griseus
RMSMLAASGPTWDQLPPFQ

SEQ ID NO: 28 - protein, 19 aa, Cricetulus griseus
SMLHMGQPDLWTFSPISVP

SEQ ID NO: 29 - protein, 18 aa, Cricetulus griseus
MSMLAASGPTWDQLPPFQ

SEQ ID NO: 30 - protein, 14 aa, Cricetulus griseus
VRSVLLDAASGQLR

SEQ ID NO: 31 - protein, 9 aa, Cricetulus griseus
QNLDPPVSR